European Patent Specification EP 3 503 915 B1, published February 21, 2024. Title: GENETICALLY ENGINEERED VIBRIO SP. AND USES THEREOF. Applicant: Synthetic Genomics, Inc. The sequence listing filed with the application follows.

SEQUENCE LISTING (28 sequences)

SEQ ID NO: 1 - DNA, 5544 bp, Vibrio natriegens
aacaactggcataaaaaaaccgcccgaaggcggttgaagttttgattaacgttattgcaatttgctgtgaacaaaagcaagaatttcttccatcaaactatcatctacttttttaaggttcagtgccagattactgcctttgcggctgtaactcgcgcgaccttttatcaaatcgactttgtctacctttggcgatggtttggctggtgataattcagtaatccaactttctaggctttctgtgacttcttttgttagacgagcaacaccttgcgctgtgctacgctgccacaagtatccgtctgttgtacggcatttatctaacaacccttgctgatgttcagggcttagattcgtaaactgcttgtgcaatttaacaatggttgggcgaccaaggtcgccaacatttggatacgcttgaagcaactctagtggtaaagaagccgcttttaacgctccacttaccaatgcctcactgcattggaacattttcgccagcgctttctggtcttctgcttcaccgctgtctaacttggcttgcatctccttgcctttttcataaagagagagaggcttgtgagcgtttgccacatcagacaggaacttagcatgattagagttaatgttgtcgccaacataaaccagaaaatcttgctcagccagaatacaagatttacgacgacgactaccgtctaatacctcaatcttgccatcttcagtgcgacggccgacggccggatactgctgaccacgctcttttaacgtaaccaatacatcggataaagcatgctcattcaagaaagattgttcgcgtgcgttatcaacaaagactgtcgtttcagactcaaccttgtcagcaggaatacgaaccaactcgaattgaacggtattctcaccagcgaccgctaactcaatggtttgcgttttttcttttgcagcggtttgcgcttcttgaggcgtagccacgcggcgtttattagttttgccaaataattttgcgtttaattcagacgttttcaaagccatttacttattacccctgattcaatgacggccaattagagtgcaatacacgctctagttcaagtgcgctcttatgaacggcgtcttgagcggttgcgagcgttttcttaccaccttcaaaatcactcacagtgagatcaaataccgtactgtaggtgtcagcacaggtttcaaacgctcgactacgcggaatggtagccatcataacttggtcacctagaagatagttcatttcagttaaaacagaaacttgcttcttattgtcgtcctcaaacatggttggcattaagcgcacaaactcaaggccattccaatcttctgggaacatttcatacactgtcggtaagtgttggaaaaagtttaccgttgaagcccagtcaagacgtttggcagcacatggaatcagcaatgcgttagaagcatacattgcattccaaactagcggatccacgtgcgggccggtatcaatcatgatgatatcgaaatcatctgcaataatgtcgataagctgctcttttaacaaacgcacgatatctaaagatgggtcttcagataaggtttgccacgcttcggcattaaacatcgcgtcttctgggaaagcagagattgacttcaagtttggatattgcgtaggtagcaatacattcttatgcaaaaactcactatcaatctcaacaccgtctggtacgttacctaacataatatcaacggcagaatagatattatcgtgttcagcgacactgatttgtgggtttaggaatagacgtaatgagccttgtggatctaagtcaatcaaacaaatacggtagcgtttatctaagttaagcgctaaacaagccgctaaatgcaccgccgacatcgatttacccgtaccacccttttggttttgtacgttgataatccacggcttattgccattgttttttttacgctcgtggaatttaggcacctcagccgcatccatcagcatatgtgcttcttctaacgtaatggaataatgattggcgttattctttgtaaattgatggccagcggcttccattttaccaatcgcgtcatcgagttttcgacgagtcaaacccgatcgggtttccatcattgccttagacattggagggaagtagttgtcacttcgctcttccaaaacaatctcaatacggtcagcttgaacttgttgtgtgagttctgctaactcatgaagattttcaatcgttttttctcttttcatgccaatttccgttgaaaggatatctgattgcaattgtacagcagtgaacaccaataacaacaaaaaggtgcacaaacattttgaataacaatcacatataaaaacaataaaatcgactcttttatgaattatggtaaaaaatatatcaaaatataatcaaacaagttcgcacaaacgctttgctaactctataaattaaaagtgttacagcgtcacacatttacattgtaaattaaaaattatacggaacgattatattgaccggctaaattacggattatgtaaaatcaacatgtttacaacaaaaaatgcagaaacggggacaagattcattcacggataccctcttgatcatgcttccaaagcatttgaggccgtttttttaatagatggaccggaaagatgatcaagagagttacttgatcatctttccgtgttatatcctacttacgaaagcatgatcatggcaaaagtaggggagtgcatgagtagatggacgttattctatgcgatcaaaccatcggaaaaatgatcaagtgaataggtttctcggaagcatgctttttactcgccattttacggacgaatgcagatatactggggcattcagagaatcaagcgtaaacaaacctcggaacgatgaaataaaaacatggtatttgataagtacggctatcatgatcatgcttcctaaatttagaacagatataggatttacacgcttagtactgatatctgatgatattttcagcacatgaataaattaccgccgaaatgagactttaacttggcattaacgctactcttgatcatcgatccggaaccaaggaggcgataaaatccatggtgtttacacctttgttgatcaagcaaacccgcatttctgtggataacctgtacaaatgtcatgatcatcgtttcaagaccattttgatcatcttttcagaaacttaatgatcatgcttacgagaggatatgatcatgctttcaagatattgttgatcatcgtttcgttatattcatgatcatggttccgaaagggatttcaataattcctttttataacaacaacttaaaatgataaaaattgccagatcaatagatcatataatcaattaagatcagaataatcaaaaagatcagttatttaaaaaacaagattttttctttatttatgatctgtttttctttattcttcggaaccatagcacaactacggctagtgtgatctggatctaaaatgatggctgatgaaaaaattctgattaaagcaccaagaagccacaaagacgggcatctttttgaagtgcacgaatcttctgcagattgggtagaacaataccaacacttcaaaggggtgaccaaaagcatcttagaattgcttaatctgatctcgttgagaggtttcagcagcaaagatggacttgtatcaaccactgaaatcgttgaagcaacagatggtcaactgactcgtgctgcgttacaacaacgattacgagcagcggtgaacattggtttatttacgcaaactccagttcgctttgaagaaggactggcaggtaaaaccatgcttcacacgtttgttaatcccaataagctcatttccgctttgggtgcaacgagcttagttactgaaaaagtccgccagaatgaaaaacaaaaacgctcaaaagcactagctcagacgcaagtaaacaaacgcttgctgacagaacatggcttaaacacgccgccgacgatgaaagatgaagcggatcaattcgtcgtctctccaactaattgggcagggatcattgaccaagctttggcgccaccacgtactcgtaagagttatcagaagtcgatggtgtcgatctctggtacgaaagcggtaatagaaactcgatcgtcaaaaaatatcatgacagtcgatgatctgatgaccttgtttgcgctgtttaccctgaccgtgcaataccatgatcatcacaaagatcagtaccatcttgatgcagctcatgtaccgaataaaacaccgctgtatatcaccgacatcctgtcattgcgtggcaaaaaggacagtggacctgctcgtgattccattcgtgacagtatcgatagaatcgaattcaccgacttccagttacatgagcttacaggccgctggttaagtgaaaacatgccggaaggttttaaaagtgatcgattccgctttctagcgcgaacgatcaccgcatcagaagaagcgccagttgagggcagcgacggtgagatccgaatcaaacctaatttgtacatattggtttgggagccgtcgttttacgaggaattactgactcgtgattacttcttcctgtttccgccagagattctgaaacaacatactttggtgttccagttatattcctttttccgtagccggatggttcgtcgccatacggattgtatgttgcttagtgaactgaatcagaagttagcgcgtaacatcgagtggcgtcgattctccatggatcttatccgggaactgaaacgattatctgatggaaaagggacggaagatctttttgttgttaacttatggggctaccacctgacgatcgaaaccatgatcgagaaaggcaaaatcatggattaccagatcgatatcaagtgtgatgttgaggaagtcttgcgttattcacgtgctcgtaccacaaacgcaggaaagcgtaacatggctcctacgctgccaaacccacttcgtaatgagatggtatccaaacaacagctagaagagctctcaggcatcattgacggcgaatttgagcctattcagcgcaaagcaccgtctcctcgtggtaatttagggcgtaggatcaagcaaagaaaacatctggttgagattaatgcagatgaaattaccattactctatccaaatatacctcaccagaggctctggaacgcagcataacggcgttatcagcaatgacagggcactcatacgcctcgattaaggaagagtgctctgagtacattgagaagcttgattggttaagagttggagatgacccattaccttatgagactctgagtaagaccgttgagctgttcaatacgcaaaatgatctcaaacatcttactattgagcgtctgattgccggtttagctgttcgtcgcaaggtctgcagacaaatttatgatggccatatggatgagatggtgtatcgagctcttgatgaaatggcgatttaacatcattcagctttatgaattgaaaccgattaatgtgactgattgattttaaatgtaaatatatatttcgataatagaaaac

SEQ ID NO: 2 - DNA, 799 bp, Artificial Sequence
  Synthetic
  misc_feature: R6Ky origin of replication
caaccatcatcgatgaattgcttcgttaatacagatgtaggtgttccacagggtagccagcagcatcctgcgatgcagatccggatgccatttcattacctctttctccgcacccgacatagatccgaagatcagcagttcaacctgttgatagtacgtactaagctctcatgtttcacgtactaagctctcatgtttaacgtactaagctctcatgtttaacgaactaaaccctcatggctaacgtactaagctctcatggctaacgtactaagctctcatgtttcacgtactaagctctcatgtttgaacaataaaattaatataaatcagcaacttaaatagcctctaaggttttaagttttataagaaaaaaaagaatatataaggcttttaaagcttttaaggtttaacggttgtggacaacaagccagggatctgccatttcattacctctttctccgcacccgacatagatccggaacataatggtgcagggcgctgacttccgcgtttccagactttacgaaacacggaaaccgaagaccattcatgttgttgctcaggtcgcagacgttttgcagcagcagtcgcttcacgttcgctcgcgtatcggtgattcattctgctaaccagtaaggcaaccccgccagcctagccgggtcctcaacgacaggagcacgatcatgcgcacccgtggccaggacccaacgctgcccgagatgcgccgcgtgcggctgctggagatggcggacgcgatggatatgttctgccaagggttggtttgcgcattcacagg

SEQ ID NO: 3 - DNA, 2727 bp, Artificial Sequence
  Synthetic
  misc_feature: tetA/tetR resistance genes + RP4 oriT
ccgtcgatctatctcatctgcgcaaggcagaacgtgaagacggccgccctggacctcgcccgcgagcgccagcgcacgaggccggcgcgcggacccgccgcggcccacgagcggacgccgcagcaggagcgccagaaggccgccagagaggccgagcgcggcgtgaggcttggacgctagggcagggcatgaaaaagcccgtagcgggcgctacggggctctgacgcggtggaaagggggaggggatgttgtctacatggctctgctgtagtgagtgggttgcgctccggcagcggtcctgatcaatcgtcaccctttctcggtccttcaacgttcctgacaacgagcctccttttcgccaatccatcgacaatcaccgcgagtccctgctcgaacgctgcgtccggaccggcttcgtcgaaggcgtctatcgcggcccgcaacagcggcgagagcggagcctgttcaacggtgccgccgcgctcgccggactcgctgtcgccggcctgctcctcaagcacggccccaacagtgaagtagctgattgtcatcagcgcattgacggcgtccccggccgaaaaacccgcctcgcagaggaagcgaagctgcgcgtcggccgtttccatctgcggtgcgcccggtcgcgtgccggcatggatgcgcgcgccatcgcggtaggcgagcagcgcctgcctgaagctgcgggcattcccagtcagaaatgagcgccagtcgtcgtcggctctcggcaccgaagtgctatgattctccgccagcatggcttcggccagtgcgtcgagcagcgcccgcttgttcctgaagtgccagtaaagcgccggctgctgaacccccaaccgttccgccagtttgcgtgtcgtcagaccgtctacgccgacctcgttcaacaggtctagggcggcacggatcactgtattcggctgcaactttgtcatgcttgacactttatcactgataaacataatatgtccaccaacttatcagtgataaagaatccgcgcgttcaatcggaccagcggaggctggtccggaggccagacgtgaaacccaacatacccctgatcgtaattctgagcactgtcgcgctcgacgctgtcggcatcggcctgattatgccggtgctgccgggcctcctgcgcgatctggttcactcgaacgacgtcaccgcccactatggcattctgctggcgctgtatgcgttggtgcaatttgcctgcgcacctgtgctgggcgcgctgtcggatcgtttcgggcggcggccaatcttgctcgtctcgctggccggcgccactgtcgactacgccatcatggcgacagcgcctttcctttgggttctctatatcgggcggatcgtggccggcatcaccggggcgactggggcggtagccggcgcttatattgccgatatcactgatggcgatgagcgcgcgcggcacttcggcttcatgagcgcctgtttcgggttcgggatggtcgcgggacctgtgctcggtgggctgatgggcggtttctccccccacgctccgttcttcgccgcggcagccttgaacggcctcaatttcctgacgggctgtttccttttgccggagtcgcacaaaggcgaacgccggccgttacgccgggaggctctcaacccgctcagcttcgttcggtgggcccggggcatgaccgtcgtcgccgccctgatggcggtcttcttcatcatgcaacttgtcggacaggtgccggccgcgctttgggtcattttcggcgaggatcgctttcactgggacgcgaccacgatcggcatttcgcttgccgcatttggcattctgcattcactcgcccaggcaatgatcaccggccctgtagccgcccggctcggcgaaaggcgggcactcatgctcggaatgattgccgacggcacaggctacatcctgcttgccttcgcgacacggggatggatggcgttcccgatcatggtcctgcttgcttcgggtggcatcggaatgccggcgctgcaagcaatgttgtccaggcaggtggatgaggaacgccaggggcagctgcaaggctcactggcggcgctcaccagcctgacctcgatcgtcggacccctcctcttcacggcgatctatgcggcttctataacaacgtggaacgggtgggcatggattgcaggcgctgccctctacttgctctgcctgccggcgctgcgtcgcgggctttggagcggcgcagggcaacgagccgatcgctgatcgtggaaacgatagggacggatctgctggcgaaagggggatgtgctgcaaggcgattaagttgggtaacgccagggttttcccagtcacgacgttgtaaaacgacggccagtgaattaattcttgaagacgaaagggcctcgtgatacgcctatttttataggttaatgtcatgataataatggtttcttagagcttacggccagcctcgcagagcaggattcccgttgagcaccgccaggtgcgaataagggacagtgaagaaggaacacccgctcgcgggtgggcctacttcacctatcctgcccggctgacgccgttggatacaccaaggaaagtctacacgaaccctttggcaaaatcctgtatatcgtgcgaaaaaggatggatataccgaaaaaatcgctataatgaccccgaagcagggttatgcagcggaaaagatccgtcgatcgacccaggtggcact

SEQ ID NO: 4 - DNA, 11285 bp, Artificial Sequence
  Synthetic
  misc_feature: pVnatCII-YACTRP-copycontrol
agcttacggccagcctcgcagagcaggattcccgttgagcaccgccaggtgcgaataagggacagtgaagaaggaacacccgctcgcgggtgggcctacttcacctatcctgcccggctgacgccgttggatacaccaaggaaagtctacacgaaccctttggcaaaatcctgtatatcgtgcgaaaaaggatggatataccgaaaaaatcgctataatgaccccgaagcagggttatgcagcggaaaagatccgtcgatcgacccaggtggcactaacaactggcataaaaaaaccgcccgaaggcggttgaagttttgattaacgttattgcaatttgctgtgaacaaaagcaagaatttcttccatcaaactatcatctacttttttaaggttcagtgccagattactgcctttgcggctgtaactcgcgcgaccttttatcaaatcgactttgtctacctttggcgatggtttggctggtgataattcagtaatccaactttctaggctttctgtgacttcttttgttagacgagcaacaccttgcgctgtgctacgctgccacaagtatccgtctgttgtacggcatttatctaacaacccttgctgatgttcagggcttagattcgtaaactgcttgtgcaatttaacaatggttgggcgaccaaggtcgccaacatttggatacgcttgaagcaactctagtggtaaagaagccgcttttaacgctccacttaccaatgcctcactgcattggaacattttcgccagcgctttctggtcttctgcttcaccgctgtctaacttggcttgcatctccttgcctttttcataaagagagagaggcttgtgagcgtttgccacatcagacaggaacttagcatgattagagttaatgttgtcgccaacataaaccagaaaatcttgctcagccagaatacaagatttacgacgacgactaccgtctaatacctcaatcttgccatcttcagtgcgacggccgacggccggatactgctgaccacgctcttttaacgtaaccaatacatcggataaagcatgctcattcaagaaagattgttcgcgtgcgttatcaacaaagactgtcgtttcagactcaaccttgtcagcaggaatacgaaccaactcgaattgaacggtattctcaccagcgaccgctaactcaatggtttgcgttttttcttttgcagcggtttgcgcttcttgaggcgtagccacgcggcgtttattagttttgccaaataattttgcgtttaattcagacgttttcaaagccatttacttattacccctgattcaatgacggccaattagagtgcaatacacgctctagttcaagtgcgctcttatgaacggcgtcttgagcggttgcgagcgttttcttaccaccttcaaaatcactcacagtgagatcaaataccgtactgtaggtgtcagcacaggtttcaaacgctcgactacgcggaatggtagccatcataacttggtcacctagaagatagttcatttcagttaaaacagaaacttgcttcttattgtcgtcctcaaacatggttggcattaagcgcacaaactcaaggccattccaatcttctgggaacatttcatacactgtcggtaagtgttggaaaaagtttaccgttgaagcccagtcaagacgtttggcagcacatggaatcagcaatgcgttagaagcatacattgcattccaaactagcggatccacgtgcgggccggtatcaatcatgatgatatcgaaatcatctgcaataatgtcgataagctgctcttttaacaaacgcacgatatctaaagatgggtcttcagataaggtttgccacgcttcggcattaaacatcgcgtcttctgggaaagcagagattgacttcaagtttggatattgcgtaggtagcaatacattcttatgcaaaaactcactatcaatctcaacaccgtctggtacgttacctaacataatatcaacggcagaatagatattatcgtgttcagcgacactgatttgtgggtttaggaatagacgtaatgagccttgtggatctaagtcaatcaaacaaatacggtagcgtttatctaagttaagcgctaaacaagccgctaaatgcaccgccgacatcgatttacccgtaccacccttttggttttgtacgttgataatccacggcttattgccattgttttttttacgctcgtggaatttaggcacctcagccgcatccatcagcatatgtgcttcttctaacgtaatggaataatgattggcgttattctttgtaaattgatggccagcggcttccattttaccaatcgcgtcatcgagttttcgacgagtcaaacccgatcgggtttccatcattgccttagacattggagggaagtagttgtcacttcgctcttccaaaacaatctcaatacggtcagcttgaacttgttgtgtgagttctgctaactcatgaagattttcaatcgttttttctcttttcatgccaatttccgttgaaaggatatctgattgcaattgtacagcagtgaacaccaataacaacaaaaaggtgcacaaacattttgaataacaatcacatataaaaacaataaaatcgactcttttatgaattatggtaaaaaatatatcaaaatataatcaaacaagttcgcacaaacgctttgctaactctataaattaaaagtgttacagcgtcacacatttacattgtaaattaaaaattatacggaacgattatattgaccggctaaattacggattatgtaaaatcaacatgtttacaacaaaaaatgcagaaacggggacaagattcattcacggataccctcttgatcatgcttccaaagcatttgaggccgtttttttaatagatggaccggaaagatgatcaagagagttacttgatcatctttccgtgttatatcctacttacgaaagcatgatcatggcaaaagtaggggagtgcatgagtagatggacgttattctatgcgatcaaaccatcggaaaaatgatcaagtgaataggtttctcggaagcatgctttttactcgccattttacggacgaatgcagatatactggggcattcagagaatcaagcgtaaacaaacctcggaacgatgaaataaaaacatggtatttgataagtacggctatcatgatcatgcttcctaaatttagaacagatataggatttacacgcttagtactgatatctgatgatattttcagcacatgaataaattaccgccgaaatgagactttaacttggcattaacgctactcttgatcatcgatccggaaccaaggaggcgataaaatccatggtgtttacacctttgttgatcaagcaaacccgcatttctgtggataacctgtacaaatgtcatgatcatcgtttcaagaccattttgatcatcttttcagaaacttaatgatcatgcttacgagaggatatgatcatgctttcaagatattgttgatcatcgtttcgttatattcatgatcatggttccgaaagggatttcaataattcctttttataacaacaacttaaaatgataaaaattgccagatcaatagatcatataatcaattaagatcagaataatcaaaaagatcagttatttaaaaaacaagattttttctttatttatgatctgtttttctttattcttcggaaccatagcacaactacggctagtgtgatctggatctaaaatgatggctgatgaaaaaattctgattaaagcaccaagaagccacaaagacgggcatctttttgaagtgcacgaatcttctgcagattgggtagaacaataccaacacttcaaaggggtgaccaaaagcatcttagaattgcttaatctgatctcgttgagaggtttcagcagcaaagatggacttgtatcaaccactgaaatcgttgaagcaacagatggtcaactgactcgtgctgcgttacaacaacgattacgagcagcggtgaacattggtttatttacgcaaactccagttcgctttgaagaaggactggcaggtaaaaccatgcttcacacgtttgttaatcccaataagctcatttccgctttgggtgcaacgagcttagttactgaaaaagtccgccagaatgaaaaacaaaaacgctcaaaagcactagctcagacgcaagtaaacaaacgcttgctgacagaacatggcttaaacacgccgccgacgatgaaagatgaagcggatcaattcgtcgtctctccaactaattgggcagggatcattgaccaagctttggcgccaccacgtactcgtaagagttatcagaagtcgatggtgtcgatctctggtacgaaagcggtaatagaaactcgatcgtcaaaaaatatcatgacagtcgatgatctgatgaccttgtttgcgctgtttaccctgaccgtgcaataccatgatcatcacaaagatcagtaccatcttgatgcagctcatgtaccgaataaaacaccgctgtatatcaccgacatcctgtcattgcgtggcaaaaaggacagtggacctgctcgtgattccattcgtgacagtatcgatagaatcgaattcaccgacttccagttacatgagcttacaggccgctggttaagtgaaaacatgccggaaggttttaaaagtgatcgattccgctttctagcgcgaacgatcaccgcatcagaagaagcgccagttgagggcagcgacggtgagatccgaatcaaacctaatttgtacatattggtttgggagccgtcgttttacgaggaattactgactcgtgattacttcttcctgtttccgccagagattctgaaacaacatactttggtgttccagttatattcctttttccgtagccggatggttcgtcgccatacggattgtatgttgcttagtgaactgaatcagaagttagcgcgtaacatcgagtggcgtcgattctccatggatcttatccgggaactgaaacgattatctgatggaaaagggacggaagatctttttgttgttaacttatggggctaccacctgacgatcgaaaccatgatcgagaaaggcaaaatcatggattaccagatcgatatcaagtgtgatgttgaggaagtcttgcgttattcacgtgctcgtaccacaaacgcaggaaagcgtaacatggctcctacgctgccaaacccacttcgtaatgagatggtatccaaacaacagctagaagagctctcaggcatcattgacggcgaatttgagcctattcagcgcaaagcaccgtctcctcgtggtaatttagggcgtaggatcaagcaaagaaaacatctggttgagattaatgcagatgaaattaccattactctatccaaatatacctcaccagaggctctggaacgcagcataacggcgttatcagcaatgacagggcactcatacgcctcgattaaggaagagtgctctgagtacattgagaagcttgattggttaagagttggagatgacccattaccttatgagactctgagtaagaccgttgagctgttcaatacgcaaaatgatctcaaacatcttactattgagcgtctgattgccggtttagctgttcgtcgcaaggtctgcagacaaatttatgatggccatatggatgagatggtgtatcgagctcttgatgaaatggcgatttaacatcattcagctttatgaattgaaaccgattaatgtgactgattgattttaaatgtaaatatatatttcgataatagaaaacgtcgacgagctcgcgagctcggacatgaggttgccccgtattcagtgtcgctgatttgtattgtctgaagttgtttttacgttaagttgatgcagatcaattaatacgatacctgcgtcataattgattatttgacgtggtttgatggcctccacgcacgttgtgatatgtagatgataatcattatcactttacgggtcctttccggtgatccgacaggttacggggcggcgacctcgcgggttttcgctatttatgaaaattttccggtttaaggcgtttccgttcttcttcgtcataacttaatgtttttatttaaaataccctctgaaaagaaaggaaacgacaggtgctgaaagcgagctttttggcctctgtcgtttcctttctctgtttttgtccgtggaatgaacaatggaagtccgagctcatcgctaataacttcgtatagcatacattatacgaagttatattcgatgcggccgcaaggggttcgcgtcagcgggtgttggcgggtgtcggggctggcttaactatgcggcatcagagcagattgtactgagagtgcaccatatgcggtgtgaaataccacacagatgcgtaaggagaaaataccgcatcaggcgccattcgccattcagctgcgcaactgttgggaagggcgatcggtgcgggcctcttcgctattacgccagctggcgaaagggggatgtgctgcaaggcgattaagttgggtaacgccagggttttcccagtcacgacgttgtaaaacgacggccagtgaattgtaatacgactcactatagggcgaattcgagctcggtacccggggatcctctagagtcgacctgcaggcatgcaagcttgagtattctatagtctcacctaaatagcttggcgtaatcatggtcatagctgtttcctgtgtgaaattgttatccgctcacaattccacacaacatacgagccggaagcataaagtgtaaagcctggggtgcctaatgagtgagctaactcacattaattgcgttgcgctcactgcccgctttccagtcgggaaacctgtcgtgccagctgcattaatgaatcggccaacgcgaaccccttgcggccgcccgggccgtcgaccaattctcatgtttgacagcttatcatcgaatttctgccattcatccgcttattatcacttattcaggcgtagcaaccaggcgtttaagggcaccaataactgccttaaaaaaattacgccccgccctgccactcatcgcagtactgttgtaattcattaagcattctgccgacatggaagccatcacaaacggcatgatgaacctgaatcgccagcggcatcagcaccttgtcgccttgcgtataatatttgcccatggtgaaaacgggggcgaagaagttgtccatattggccacgtttaaatcaaaactggtgaaactcacccagggattggctgagacgaaaaacatattctcaataaaccctttagggaaataggccaggttttcaccgtaacacgccacatcttgcgaatatatgtgtagaaactgccggaaatcgtcgtggtattcactccagagcgatgaaaacgtttcagtttgctcatggaaaacggtgtaacaagggtgaacactatcccatatcaccagctcaccgtctttcattgccatacgaaattccggatgagcattcatcaggcgggcaagaatgtgaataaaggccggataaaacttgtgcttatttttctttacggtctttaaaaaggccgtaatatccagctgaacggtctggttataggtacattgagcaactgactgaaatgcctcaaaatgttctttacgatgccattgggatatatcaacggtggtatatccagtgatttttttctccattttagcttccttagctcctgaaaatctcgataactcaaaaaatacgcccggtagtgatcttatttcattatggtgaaagttggaacctcttacgtgccgatcaacgtctcattttcgccaaaagttggcccagggcttcccggtatcaacagggacaccaggatttatttattctgcgaagtgatcttccgtcacaggtatttattcgcgataagctcatggagcggcgtaaccgtcgcacaggaaggacagagaaagcgcggatctgggaagtgacggacagaacggtcaggacctggattggggaggcggttgccgccgctgctgctgacggtgtgacgttctctgttccggtcacaccacatacgttccgccattcctatgcgatgcacatgctgtatgccggtataccgctgaaagttctgcaaagcctgatgggacataagtccatcagttcaacggaagtctacacgaaggtttttgcgctggatgtggctgcccggcaccgggtgcagtttgcgatgccggagtctgatgcggttgcgatgctgaaacaattatcctgagaataaatgccttggcctttatatggaaatgtggaactgagtggatatgctgtttttgtctgttaaacagagaagctggctgttatccactgagaagcgaacgaaacagtcgggaaaatctcccattatcgtagagatccgcattattaatctcaggagcctgtgtagcgtttataggaagtagtgttctgtcatgatgcctgcaagcggtaacgaaaacgatttgaatatgccttcaggaacaatagaaatcttcgtgcggtgttacgttgaagtggagcggattatgtcagcaatggacagaacaacctaatgaacacagaaccatgatgtggtctgtccttttacagccagtagtgctcgccgcagtcgagcgacagggcgaagccctcgagctggttgccctcgccgctgggctggcggccgtctatggccctgcaaacgcgccagaaacgccgtcgaagccgtgtgcgagacaccgcggccggccgccggcgttgtggatacctcgcggaaaacttggccctcactgacagatgaggggcggacgttgacacttgaggggccgactcacccggcgcggcgttgacagatgaggggcaggctcgatttcggccggcgacgtggagctggccagcctcgcaaatcggcgaaaacgcctgattttacgcgagtttcccacagatgatgtggacaagcctggggataagtgccctgcggtattgacacttgaggggcgcgactactgacagatgaggggcgcgatccttgacacttgaggggcagagtgctgacagatgaggggcgcacctattgacatttgaggggctgtccacaggcagaaaatccagcatttgcaagggtttccgcccgtttttcggccaccgctaacctgtcttttaacctgcttttaaaccaatatttataaaccttgtttttaaccagggctgcgccctgtgcgcgtgaccgcgcacgccgaaggggggtgcccccccttctcgaaccctcccggcagttcgctcgctatgctcggttacacggctgcggcgagcatcacgtgctataaaaataattataatttaaattttttaatataaatatataaattaaaaatagaaagtaaaaaaagaaattaaagaaaaaatagtttttgttttccgaagatgtaaaagactctagggggatcgccaacaaatactaccttttatcttgctcttcctgctctcaggtattaatgccgaattgtttcatcttgtctgtgtagaagaccacacacgaaaatcctgtgattttacattttacttatcgttaatcgaatgtatatctatttaatctgcttttcttgtctaataaatatatatgtaaagtacgctttttgttgaaattttttaaacctttgtttatttttttttcttcattccgtaactcttctaccttctttatttactttctaaaatccaaatacaaaacataaaaataaataaacacagagtaaattcccaaattattccatcattaaaagatacgaggcgcgtgtaagttacaggcaagcgatccgtcctaagaaaccattattatcatgacattaacctataaaaataggcgtatcacgaggccctttcgtctcgcgcgtttcggtgatgacggtgaaaacctctgacacatgcagctcccggagacggtcacagcttgtctgtaagcggatgccgggagcagacaagcccgtcagggcgcgtcagcgggtgttggcgggtgtcggggctggcttaactatgcggcatcagagcagattgtactgagagtgcaccataaacgacattactatatatataatataggaagcatttaatagacagcatcgtaatatatgtgtactttgcagttatgacgccagatggcagtagtggaagatattctttattgaaaaatagcttgtcaccttacgtacaatcttgatccggagcttttctttttttgccgattaagaattaattcggtcgaaaaaagaaaaggagagggccaagagggagggcattggtgactattgagcacgtgagtatacgtgattaagcacacaaaggcagcttggagtatgtctgttattaatttcacaggtagttctggtccattggtgaaagtttgcggcttgcagagcacagaggccgcagaatgtgctctagattccgatgctgacttgctgggtattatatgtgtgcccaatagaaagagaacaattgacccggttattgcaaggaaaatttcaagtcttgtaaaagcatataaaaatagttcaggcactccgaaatacttggttggcgtgtttcgtaatcaacctaaggaggatgttttggctctggtcaatgattacggcattgatatcgtccaactgcatggagatgagtcgtggcaagaataccaagagttcctcggtttgccagttattaaaagactcgtatttccaaaagactgcaacatactactcagtgcagcttcacagaaacctcattcgtttattcccttgtttgattcagaagcaggtgggacaggtgaacttttggattggaactcgatttctgactgggttggaaggcaagagagccccgaaagcttacattttatgttagctggtggactgacgccagaaaatgttggtgatgcgcttagattaaatggcgttattggtgttgatgtaagcggaggtgtggagacaaatggtgtaaaagactctaacaaaatagcaaatttcgtcaaaaatgctaagaaataggttattactgagtagtatttatttaagtattgtttgtgcacttgcctatgcggtgtgaaataccgcacagatgcgtaaggagaaaataccgcatcaggaaattgtaaacgttaatattttgttaaaattcgcgttaaatttttgttaaatcagctcattttttaaccaataggccgaaatcggcaaaatcgctagtgataataagtgactgaggtatgtgctcttcttat

SEQ ID NO: 5 - DNA, 1217 bp, Artificial Sequence
  Synthetic
  misc_feature: araC-araBAD promoter fragment
ttatgacaacttgacggctacatcattcactttttcttcacaaccggcacggaactcgctcgggctggccccggtgcattttttaaatacccgcgagaaatagagttgatcgtcaaaaccaacattgcgaccgacggtggcgataggcatccgggtggtgctcaaaagcagcttcgcctggctgatacgttggtcctcgcgccagcttaagacgctaatccctaactgctggcggaaaagatgtgacagacgcgacggcgacaagcaaacatgctgtgcgacgctggcgatatcaaaattgctgtctgccaggtgatcgctgatgtactgacaagcctcgcgtacccgattatccatcggtggatggagcgactcgttaatcgcttccatgcgccgcagtaacaattgctcaagcagatttatcgccagcagctccgaatagcgcccttccccttgcccggcgttaatgatttgcccaaacaggtcgctgaaatgcggctggtgcgcttcatccgggcgaaagaaccccgtattggcaaatattgacggccagttaagccattcatgccagtaggcgcgcggacgaaagtaaacccactggtgataccattcgcgagcctccggatgacgaccgtagtgatgaatctctcctggcgggaacagcaaaatatcacccggtcggcaaacaaattctcgtccctgatttttcaccaccccctgaccgcgaatggtgagattgagaatataacctttcattcccagcggtcggtcgataaaaaaatcgagataaccgttggcctcaatcggcgttaaacccgccaccagatgggcattaaacgagtatcccggcagcaggggatcattttgcgcttcagccatacttttcatactcccgccattcagagaagaaaccaattgtccatattgcatcagacattgccgtcactgcgtcttttactggctcttctcgctaaccaaaccggtaaccccgcttattaaaagcattctgtaacaaagcgggaccaaagccatgacaaaaacgcgtaacaaaagtgtctataatcacggcagaaaagtccacattgattatttgcacggcgtcacactttgctatgccatagcatttttatccataagattagcggatcctacctgacgctttttatcgcaactctctactgtttctccatacccgtttttttggatggagtgaaacg

SEQ ID NO: 6 - DNA, 1937 bp, Artificial Sequence
  Synthetic
  misc_feature: lac operon regulatory elements and lacI protein
ttatttgatttcaattttgtcccactccctgcctctgtcatcacgatactgtgatgccatggtgtccgacttatgcccgagaagatgttgagcaaacttatcgcttatctgcttctcatagagtcttgcagacaaactgcgcaactcgtgaaaggtaggcggatccagatcccggacaccatcgaatggcgcaaaacctttcgcggtatggcatgatagcgcccggaagagagtcaattcagggtggtgaatgtgaaaccagtaacgttatacgatgtcgcagagtatgccggtgtctcttatcagaccgtttcccgcgtggtgaaccaggccagccacgtttctgcgaaaacgcgggaaaaagtggaagcggcgatggcggagctgaattacattcccaaccgcgtggcacaacaactggcgggcaaacagtcgttgctgattggcgttgccacctccagtctggccctgcacgcgccgtcgcaaattgtcgcggcgattaaatctcgcgccgatcaactgggtgccagcgtggtggtgtcgatggtagaacgaagcggcgtcgaagcctgtaaagcggcggtgcacaatcttctcgcgcaacgcgtcagtgggctgatcattaactatccgctggatgaccaggatgccattgctgtggaagctgcctgcactaatgttccggcgttatttcttgatgtctctgaccagacacccatcaacagtattattttctcccatgaagacggtacgcgactgggcgtggagcatctggtcgcattgggtcaccagcaaatcgcgctgttagcgggcccattaagttctgtctcggcgcgtctgcgtctggctggctggcataaatatctcactcgcaatcaaattcagccgatagcggaacgggaaggcgactggagtgccatgtccggttttcaacaaaccatgcaaatgctgaatgagggcatcgttcccactgcgatgctggttgccaacgatcagatggcgctgggcgcaatgcgcgccattaccgagtccgggctgcgcgttggtgcggatatctcggtagtgggatacgacgataccgaagacagctcatgttatatcccgccgttaaccaccatcaaacaggattttcgcctgctggggcaaaccagcgtggaccgcttgctgcaactctctcagggccaggcggtgaagggcaatcagctgttgcccgtctcactggtgaaaagaaaaaccaccctggcgcccaatacgcaaaccgcctctccccgcgcgttggccgattcattaatgcagctggcacgacaggtttcccgactggaaagcgggcagtgagcgcaacgcaattaatgtaagttagctcactcattaggcaccccaggctttacactttatgcttccggctcgtataatgtgtggaattgtgagcggataacaatttcacacaggaaacagctatgaccatgattacggattcactggccgtcgttttacaacgtcgtgactgggaaaaccctggcgttacccaacttaatcgccttgcagcacatccccctttcgccagctggcgtaatagcgaagaggcccgcaccgatcgcccttcccaacagttgcgcagcctgaatggcgaatggcgctttgcctggtttccggcaccagaagcggtgccggaaagctggctggagtgcgatcttcctgaggccgatactgtcgtcgtcccctcaaactggcagatgcacggttacgatgcgcccatctacaccaacgtgacctatcccattacggtcaatccgccgtttgttcccacggagaatccgacgggttgttactcgctcacatttaatgttgatgaaagctggctacaggaaggccagacgcgaattatttttgatggcgtcgggatctgatccggatttactaactggaagaggcactaa

SEQ ID NO: 7 - DNA, 2652 bp, Artificial Sequence
  Synthetic
  misc_feature: T7 RNA polymerase gene
atgaacacgattaacatcgctaagaacgacttctctgacatcgaactggctgctatcccgttcaacactctggctgaccattacggtgagcgtttagctcgcgaacagttggcccttgagcatgagtcttacgagatgggtgaagcacgcttccgcaagatgtttgagcgtcaacttaaagctggtgaggttgcggataacgctgccgccaagcctctcatcactaccctactccctaagatgattgcacgcatcaacgactggtttgaggaagtgaaagctaagcgcggcaagcgcccgacagccttccagttcctgcaagaaatcaagccggaagccgtagcgtacatcaccattaagaccactctggcttgcctaaccagtgctgacaatacaaccgttcaggctgtagcaagcgcaatcggtcgggccattgaggacgaggctcgcttcggtcgtatccgtgaccttgaagctaagcacttcaagaaaaacgttgaggaacaactcaacaagcgcgtagggcacgtctacaagaaagcatttatgcaagttgtcgaggctgacatgctctctaagggtctactcggtggcgaggcgtggtcttcgtggcataaggaagactctattcatgtaggagtacgctgcatcgagatgctcattgagtcaaccggaatggttagcttacaccgccaaaatgctggcgtagtaggtcaagactctgagactatcgaactcgcacctgaatacgctgaggctatcgcaacccgtgcaggtgcgctggctggcatctctccgatgttccaaccttgcgtagttcctcctaagccgtggactggcattactggtggtggctattgggctaacggtcgtcgtcctctggcgctggtgcgtactcacagtaagaaagcactgatgcgctacgaagacgtttacatgcctgaggtgtacaaagcgattaacattgcgcaaaacaccgcatggaaaatcaacaagaaagtcctagcggtcgccaacgtaatcaccaagtggaagcattgtccggtcgaggacatccctgcgattgagcgtgaagaactcccgatgaaaccggaagacatcgacatgaatcctgaggctctcaccgcgtggaaacgtgctgccgctgctgtgtaccgcaaggacaaggctcgcaagtctcgccgtatcagccttgagttcatgcttgagcaagccaataagtttgctaaccataaggccatctggttcccttacaacatggactggcgcggtcgtgtttacgctgtgtcaatgttcaacccgcaaggtaacgatatgaccaaaggactgcttacgctggcgaaaggtaaaccaatcggtaaggaaggttactactggctgaaaatccacggtgcaaactgtgcgggtgtcgataaggttccgttccctgagcgcatcaagttcattgaggaaaaccacgagaacatcatggcttgcgctaagtctccactggagaacacttggtgggctgagcaagattctccgttctgcttccttgcgttctgctttgagtacgctggggtacagcaccacggcctgagctataactgctcccttccgctggcgtttgacgggtcttgctctggcatccagcacttctccgcgatgctccgagatgaggtaggtggtcgcgcggttaacttgcttcctagtgaaaccgttcaggacatctacgggattgttgctaagaaagtcaacgagattctacaagcagacgcaatcaatgggaccgataacgaagtagttaccgtgaccgatgagaacactggtgaaatctctgagaaagtcaagctgggcactaaggcactggctggtcaatggctggcttacggtgttactcgcagtgtgactaagcgttcagtcatgacgctggcttacgggtccaaagagttcggcttccgtcaacaagtgctggaagataccattcagccagctattgattccggcaagggtctgatgttcactcagccgaatcaggctgctggatacatggctaagctgatttgggaatctgtgagcgtgacggtggtagctgcggttgaagcaatgaactggcttaagtctgctgctaagctgctggctgctgaggtcaaagataagaagactggagagattcttcgcaagcgttgcgctgtgcattgggtaactcctgatggtttccctgtgtggcaggaatacaagaagcctattcagacgcgcttgaacctgatgttcctcggtcagttccgcttacagcctaccattaacaccaacaaagatagcgagattgatgcacacaaacaggagtctggtatcgctcctaactttgtacacagccaagacggtagccaccttcgtaagactgtagtgtgggcacacgagaagtacggaatcgaatcttttgcactgattcacgactccttcggtaccattccggctgacgctgcgaacctgttcaaagcagtgcgcgaaactatggttgacacatatgagtcttgtgatgtactggctgatttctacgaccagttcgctgaccagttgcacgagtctcaattggacaaaatgccagcacttccggctaaaggtaacttgaacctccgtgacatcttagagtcggacttcgcgttcgcgtaa

SEQ ID NO: 8 - protein, 37 aa, Vibrio natriegens
MRILLTEVSKMRSTKMKAGVPILGILMGTAASQLAFA

SEQ ID NO: 9 - protein, 27 aa, Vibrio natriegens
MRSTKMKAGVPILGILMGTAASQLAFA

SEQ ID NO: 10 - protein, 25 aa, Vibrio natriegens
MQMKTMKSKLAVALIAAGLSFNSLA

SEQ ID NO: 11 - protein, 50 aa, Vibrio natriegens
MRNNQLTLALKKIKKGIRKGYPKLRKGSGLIMKKTLLALAVATVSTSALA

SEQ ID NO: 12 - protein, 19 aa, Vibrio natriegens
MKKTLLALAVATVSTSALA

SEQ ID NO: 13 - protein, 22 aa, Vibrio natriegens
MKKLSAVALGTLVALGSFGAHA

SEQ ID NO: 14 - protein, 26 aa, Vibrio natriegens
MELRMKKVSVIAAAVAASLAAGSAFA

SEQ ID NO: 15 - protein, 22 aa, Vibrio natriegens
MKKVSVIAAAVAASLAAGSAFA

SEQ ID NO: 16 - protein, 21 aa, Vibrio natriegens
MKKTLIALSVSAAAMATGVNA

SEQ ID NO: 17 - protein, 32 aa, Vibrio natriegens
MQSIQGNIMNKVAIAVAAVVAGGSALLNTAQA

SEQ ID NO: 18 - protein, 24 aa, Vibrio natriegens
MAFNKLLKVGAIAAAVMGAGAVNA

SEQ ID NO: 19 - protein, 26 aa, Vibrio natriegens
MKKPLLALTVLSLSLSSIFTPIQATA

SEQ ID NO: 20 - protein, 21 aa, Vibrio natriegens
MKKVLTLSALACATLAPTAMA

SEQ ID NO: 21 - protein, 21 aa, Vibrio natriegens
MKKWLLAATLAATAVSGAVQA

SEQ ID NO: 22 - protein, 22 aa, Vibrio natriegens
MMKNWIKVAVAAIALSAATVQA

SEQ ID NO: 23 - protein, 29 aa, Vibrio natriegens
MNTQVKKPSFMPSILAAAVVTAFSGQANA

SEQ ID NO: 24 - protein, 20 aa, Vibrio natriegens
MKKLAAVISASLLMASAAQA

SEQ ID NO: 25 - protein, 24 aa, Vibrio natriegens
MNCSHKFKLTAIAMMVGSSMSANA

SEQ ID NO: 26 - protein, 25 aa, Vibrio natriegens
MNKLLTLTPLAVAIGSSLVVPSAVA

SEQ ID NO: 27 - protein, 21 aa, Vibrio natriegens
MKKTICSLAVVAALVSPSVFA

SEQ ID NO: 28 - protein, 33 aa, Vibrio natriegens
MAITRRSFLKGVATTSAASVIGPSLLASASAKA